European Patent Specification EP 3 704 262 B1, published March 20, 2024. Title: Multiplexed Analysis of Materials for Tissue Delivery. Applicant: Georgia Tech Research Corporation Dahlman, James Sago, Cory Lokugamage, Melissa. The sequence listing filed with the application follows.

SEQUENCE LISTING (11 sequences)

SEQ ID NO: 1 - DNA, 58 bp, Artificial Sequence
  Synthetic
  misc_feature (32)..(38): n is A, C, G, or T
agacgtgtgctcttccgatctgagggtacttnnnnnnnagatcggaagagcgtcgtgt

SEQ ID NO: 2 - DNA, 21 bp, Artificial Sequence
  Synthetic
  misc_feature (5)..(5): n is 2'-O-Methylcytosine
  misc_feature (8)..(8): n is 2'-O-Methyluridine
  misc_feature (9)..(9): n is 2'-O-Methylcytosine
  misc_feature (10)..(10): n is 2'-O-Methyluridine
  misc_feature (11)..(11): n is 2'-O-Methylcytosine
  misc_feature (14)..(14): n is 2'-O-Methylcytosine
  misc_feature (15)..(18): n is 2'-O-Methyluridine
  misc_feature (19)..(19): n is 2'-O-Methylcytosine
  misc_feature (20)..(20): n is deoxy-T
  misc_feature (21)..(21): n is phosphorothioate deoxy-T
agganggnnnnaannnnnnnn

SEQ ID NO: 3 - RNA, 21 nt, Artificial Sequence
  Synthetic
  misc_feature (8)..(8): n is 2'-O-Methyluridine
  misc_feature (20)..(20): n is deoxy-T
  misc_feature (21)..(21): n is phosphorothioate deoxy-T
gaaaagungagaccguccunn

SEQ ID NO: 4 - RNA, 21 nt, Artificial Sequence
  Synthetic
  misc_feature (2)..(2): n is 2'-O-Methylcytosine
  misc_feature (4)..(4): n is 2'-O-Methyluridine
  misc_feature (9)..(9): n is 2'-O-Methylcytosine
  misc_feature (12)..(12): n is 2'-O-Methylcytosine
  misc_feature (18)..(18): n is 2'-O-Methyluridine
  misc_feature (20)..(20): n is deoxy-T
  misc_feature (21)..(21): n is phosphorothioate deoxy-T
anangaagnagnacgacnunn

SEQ ID NO: 5 - RNA, 21 nt, Artificial Sequence
  Synthetic
  misc_feature (20)..(20): n is deoxy-T
  misc_feature (21)..(21): n is phosphorothioate deoxy-T
aagucgugcugcuucaugunn

SEQ ID NO: 6 - RNA, 100 nt, Artificial Sequence
  Synthetic
  misc_feature (1)..(1): n is 2'-O-Methylguanosine with phosphorothioate linkage
  misc_feature (2)..(2): n is 2'-O-Methylcytosine with phosphorothioate linkage
  misc_feature (3)..(3): n is 2'-O-Methyluridine with phosphorothioate linkage
  misc_feature (97)..(99): n is 2'-O-Methyluridine with phosphorothioate linkage
nnnuaccugggcuguagaacguuuuagagcuagaaauagcaaguuaaaauaaggcuaguccguuaucaacuugaaaaaguggcaccgagucggugcnnnu

SEQ ID NO: 7 - RNA, 100 nt, Artificial Sequence
  Synthetic
  misc_feature (1)..(1): n is 2'-O-Methyladenosine with phosphorothioate linkage
  misc_feature (2)..(2): n is 2'-O-Methyladenosine with phosphorothioate linkage
  misc_feature (3)..(3): n is 2'-O-Methylguanosine with phosphorothioate linkage
  misc_feature (97)..(99): n is 2'-O-Methyluridine with phosphorothioate linkage
nnnacggacaggcaccuacgguuuuagagcuagaaauagcaaguuaaaauaaggcuaguccguuaucaacuugaaaaaguggcaccgagucggugcnnnu

SEQ ID NO: 8 - DNA, 84 bp, Artificial Sequence
  Synthetic
  misc_feature (24)..(24): n is A, T, G, or C
  misc_feature (25)..(25): n is A, T, or C
  misc_feature (26)..(26): n is A, T, G, or C
  misc_feature (27)..(27): n is A or T
  misc_feature (54)..(54): n is A, T, G, or C
  misc_feature (55)..(55): n is A or T
  misc_feature (56)..(56): n is A, T, G, or C
  misc_feature (57)..(57): n is A, T, or C
  misc_feature (58)..(58): n is an 8nt barcode sequence
  misc_feature (59)..(59): n is A, T, G, or C
  misc_feature (60)..(60): n is A or T
  misc_feature (61)..(61): n is A, T, or C
  misc_feature (66)..(66): n is A, T, G, or C
  misc_feature (67)..(67): n is A or T
  misc_feature (68)..(68): n is A, T, or C
gatgctctcatacgaactcgtccnnnncctgctagtccacgtccatgtccaccnnnnnnnngtggttagtcgagcagagactag

SEQ ID NO: 9 - DNA, 70 bp, Artificial Sequence
  Synthetic
aatgatacggcgaccaccgagatctacactaaggccaacactctttccctacacgacgctcttccgatct

SEQ ID NO: 10 - DNA, 33 bp, Artificial Sequence
  Synthetic
tgactggagttcagacgtgtgctcttccgatct

SEQ ID NO: 11 - DNA, 54 bp, Artificial Sequence
  Synthetic
caagcagaagacggcatacgagatatagagaggtgactggagttcagacgtgtg